European Patent Application EP 4 257 183 A1, published October 11, 2023. Title: Prebiotic composition for growing a butyrate-producing bacterium. Applicant: MORINAGA MILK INDUSTRY CO., LTD. The sequence listing filed with the application follows.

SEQUENCE LISTING (4 sequences)

SEQ ID NO: 1 - DNA, 31 bp, Artificial Sequence
  Tru357Fprimer
cgctcttccgatctctgtacggragcagcag

SEQ ID NO: 2 - DNA, 37 bp, Artificial Sequence
  Tru806Rprimer
cgctcttccgatctgacggactachvgggtwtctaat

SEQ ID NO: 3 - DNA, 73 bp, Artificial Sequence
  Barcode Fprimer
  misc_feature (30)..(37): n is a, c, g, or t
aatgatacggcgaccaccgagatctacacnnnnnnnnacactctttccctacacgacgctcttccgatctctg

SEQ ID NO: 4 - DNA, 69 bp, Artificial Sequence
  Barcode Rprimer
  misc_feature (25)..(32): n is a, c, g, or t
caagcagaagacggcatacgagatnnnnnnnngtgactggagttcagacgtgtgctcttccgatctgac